European Patent Specification EP 4 063 499 B1, published December 11, 2024. Title: Novel mycothione reductase variant and a method for producing L-lysine using the same. Applicant: CJ CheilJedang Corporation. The sequence listing filed with the application follows.

SEQUENCE LISTING (10 sequences)

SEQ ID NO: 1 - protein, 465 aa, Artificial Sequence
  (P358S)_mycothione reductase
MSEQPASIKHYDLIIIGTGSGNSIPGPEFDDKSIAIVEKGAFGGTCLNVGCIPTKMYVYAADIAQEIQESARLGIDATVNSVDWPSIVSRVFDKRIDLIAQGGEAYRRGPETPNIDVYDMHASFVDSKTISTGIAGQEQLISGTDIVIATGSRPYIPEAIAESGARYYTNEDIMRLAQQPESLVIVGGGFIALEFAHVFEALGTKVTILNRSDVLLREADADISAKILELSKKRFDVRLSTAVTAVHNKADGGVKISTDTGDDIEADILLVATGRTPNGNQMNLDAAGIEMNGRSIKVDEFGRTSVEGVWALGDVSSPYKLKHVANAEMRAIKHNLANPNDLQKMPHDFVPSAVFTNSQISQVGMTEQEAREAGLDITVKIQNYSDVAYGWAMEDKDGFVKLIADKDTGKLVGAHIIGAQASTLIQQLITVMAFGIDAREAATKQYWIHPALPEVIENALLGLEF

SEQ ID NO: 2 - DNA, 1398 bp, Artificial Sequence
  (P358S)_NCgl1928
atgtctgagcagccagcttccattaagcattatgacctcatcatcattggtaccggctctggaaactccattcctggaccagagtttgatgataaatcaattgccatcgtggaaaagggtgctttcggcggaacttgcctcaatgtgggctgcatccctaccaagatgtacgtttacgctgcggatatcgctcaagaaattcaggagtctgctcgcctgggtatcgatgcgacggtcaacagcgtggattggccttccatcgtcagccgcgttttcgacaagcgcatcgacctcatcgcgcaaggcggcgaggcttatcgacgtggccccgaaactccaaacatcgatgtgtatgacatgcacgcatcgtttgttgattccaagacaatctccactggtattgccggccaagaacagctgatcagcggtactgacattgtaatcgcaaccggctcccgcccttacatccctgaagctattgcagagtccggcgcacgctactacaccaacgaagacatcatgcgcctggcacagcagcctgaatctttggtgattgttggtggcggtttcatcgctttggaatttgctcacgtttttgaagcgcttggcaccaaggtcaccatcctcaaccgctctgacgtgctgctgcgcgaggcagatgcagacatctccgcgaaaatcctcgagctttccaaaaagcgtttcgacgtccgcctcagcactgcggtcaccgcagtacacaacaaggccgacggcggcgtgaagatctccaccgacaccggcgacgacatcgaggcagatattttgctcgttgccactggtcgcacccctaacggcaaccaaatgaacttggacgccgcaggcatcgagatgaacggtcgttccatcaaggttgatgaattcggtcgcaccagtgttgaaggcgtgtgggcgcttggcgatgtctcctccccttacaagctcaagcacgtagccaatgcggaaatgcgagcaatcaagcacaaccttgccaaccctaatgacctgcagaagatgccacatgatttcgtgccatcagctgttttcaccaactctcagatctcgcaggtcggcatgactgagcaggaggcgcgtgaagctggcctcgacatcactgtgaagatccagaactactctgatgtggcttatggctgggccatggaagataaggatggattcgttaagctcattgccgataaggacaccggcaagttggtcggcgcgcacatcattggtgctcaagcctcaacactgatccagcaactgatcactgtcatggcatttggaatcgatgcacgagaagctgcaaccaagcagtactggattcaccctgctcttccagaagtcatcgaaaacgctcttctggggctagagttttag

SEQ ID NO: 3 - protein, 465 aa, Artificial Sequence
  (WT)_mycothione reductase
MSEQPASIKHYDLIIIGTGSGNSIPGPEFDDKSIAIVEKGAFGGTCLNVGCIPTKMYVYAADIAQEIQESARLGIDATVNSVDWPSIVSRVFDKRIDLIAQGGEAYRRGPETPNIDVYDMHASFVDSKTISTGIAGQEQLISGTDIVIATGSRPYIPEAIAESGARYYTNEDIMRLAQQPESLVIVGGGFIALEFAHVFEALGTKVTILNRSDVLLREADADISAKILELSKKRFDVRLSTAVTAVHNKADGGVKISTDTGDDIEADILLVATGRTPNGNQMNLDAAGIEMNGRSIKVDEFGRTSVEGVWALGDVSSPYKLKHVANAEMRAIKHNLANPNDLQKMPHDFVPSAVFTNPQISQVGMTEQEAREAGLDITVKIQNYSDVAYGWAMEDKDGFVKLIADKDTGKLVGAHIIGAQASTLIQQLITVMAFGIDAREAATKQYWIHPALPEVIENALLGLEF

SEQ ID NO: 4 - DNA, 1398 bp, Artificial Sequence
  (WT)_NCgl1928
atgtctgagcagccagcttccattaagcattatgacctcatcatcattggtaccggctctggaaactccattcctggaccagagtttgatgataaatcaattgccatcgtggaaaagggtgctttcggcggaacttgcctcaatgtgggctgcatccctaccaagatgtacgtttacgctgcggatatcgctcaagaaattcaggagtctgctcgcctgggtatcgatgcgacggtcaacagcgtggattggccttccatcgtcagccgcgttttcgacaagcgcatcgacctcatcgcgcaaggcggcgaggcttatcgacgtggccccgaaactccaaacatcgatgtgtatgacatgcacgcatcgtttgttgattccaagacaatctccactggtattgccggccaagaacagctgatcagcggtactgacattgtaatcgcaaccggctcccgcccttacatccctgaagctattgcagagtccggcgcacgctactacaccaacgaagacatcatgcgcctggcacagcagcctgaatctttggtgattgttggtggcggtttcatcgctttggaatttgctcacgtttttgaagcgcttggcaccaaggtcaccatcctcaaccgctctgacgtgctgctgcgcgaggcagatgcagacatctccgcgaaaatcctcgagctttccaaaaagcgtttcgacgtccgcctcagcactgcggtcaccgcagtacacaacaaggccgacggcggcgtgaagatctccaccgacaccggcgacgacatcgaggcagatattttgctcgttgccactggtcgcacccctaacggcaaccaaatgaacttggacgccgcaggcatcgagatgaacggtcgttccatcaaggttgatgaattcggtcgcaccagtgttgaaggcgtgtgggcgcttggcgatgtctcctccccttacaagctcaagcacgtagccaatgcggaaatgcgagcaatcaagcacaaccttgccaaccctaatgacctgcagaagatgccacatgatttcgtgccatcagctgttttcaccaaccctcagatctcgcaggtcggcatgactgagcaggaggcgcgtgaagctggcctcgacatcactgtgaagatccagaactactctgatgtggcttatggctgggccatggaagataaggatggattcgttaagctcattgccgataaggacaccggcaagttggtcggcgcgcacatcattggtgctcaagcctcaacactgatccagcaactgatcactgtcatggcatttggaatcgatgcacgagaagctgcaaccaagcagtactggattcaccctgctcttccagaagtcatcgaaaacgctcttctggggctagagttttag

SEQ ID NO: 5 - DNA, 40 bp, Artificial Sequence
  NCgl1928_1F
tgaattcgagctcggtaccctgaatctttggtgattgttg

SEQ ID NO: 6 - DNA, 33 bp, Artificial Sequence
  NCgl1928_2R
acctgcgagatctgagagttggtgaaaacagct

SEQ ID NO: 7 - DNA, 33 bp, Artificial Sequence
  NCgl1928_3F
agctgttttcaccaactctcagatctcgcaggt

SEQ ID NO: 8 - DNA, 40 bp, Artificial Sequence
  NCgl1928_4R
gtcgactctagaggatccccaagtctatatgtatttcctt

SEQ ID NO: 9 - DNA, 20 bp, Artificial Sequence
  NCgl1928_5F
tgaatctttggtgattgttg

SEQ ID NO: 10 - DNA, 20 bp, Artificial Sequence
  NCgl1928_6R
aagtctatatgtatttcctt